European Patent Specification EP 3 801 057 B1, published December 10, 2025. Title: USE OF PEPTIDYLARGININE DEIMINASE TO OBTAIN IMPROVED SWEET PROTEIN. Applicant: DSM IP Assets B.V. The sequence listing filed with the application follows.

SEQUENCE LISTING (1 sequence)

SEQ ID NO: 1 - protein, 640 aa, Fusarium graminearum
MHLLNGKTAAVALALLNSCNALKVTILADTNRDGKVDNNDINGKSTWTNNRGALILPNIGDTGSRCAKQWGPSVDIQGDESYLDKCNDASDNVQRNPKYLASLKTLPLTTLSATAKGSIIIADKTGASKVRIFVKQSGKWNYVAADHVFTAKELKSGLELGVDARDVRRPQDWNGYAKIQFTVTDGKTKATDAVAVRVAPVLTHHHGQHAQRIFTTGVNEAGVNKVQETFIADILRNVAGAGIKEPVFQFHNQDIWTQDFFEPGYASIPGPNGPVSIRIMIRSAQSSRRSGRDAFHDLRNDQVGAVQHPGDGDSIDSTGNLETIPPYSHNGKSFPVGRTIMGAWDGRAPLMVEFLKAQQVQEPLILDTSWLYVGHVDEFIQFLPSNNKLGWVIMVADPMKGVDLLKKAVKTGHGKVKAVSRPLSADEKKEQLCLPRQTIAEALKFKSFDAINKHSAERIQANLDIIKRETGITDEDIHRVPALFYYTQSNSWLCPGETAEDDSAQPQKAASNSGITMKTSQGGPGFKAKSIVEAATPGKSIQRRVIDPATQVTALYPGSVNGLVMTDTKILAPSPWGPVINKQDIFAAAVSQVYTNAGYNVTYQDDWFSHFKLQGDVHCGSNSWREIPKKWWDSLRVNNY